European Patent Application EP 4 324 927 A1, published February 21, 2024. Title: ENZYME COMPOSITION FOR PREPARING beta-NICOTINAMIDE MONONUCLEOTIDE, AND APPLICATION THEREOF. Applicant: SHENZHEN READLINE BIOTECH CO., LTD. The sequence listing filed with the application follows.

SEQUENCE LISTING (13 sequences)

SEQ ID NO: 1 - protein, 289 aa, Artificial Sequence
MANGYTYEDYQDTAKWLLSHTEQRPQVAVICGSGLGGLVNKLTQAQTFDYSEIPNFPESTVPGHAGRLVFGILNGRACVMMQGRFHMYEGYPFWKVTFPVRVFRLLGVETLVVTNAAGGLNPNFEVGDIMLIRDHINLPGFSGENPLRGPNEERFGVRFPAMSDAYDRDMRQKAHSTWKQMGEQRELQEGTYVMLGGPNFETVAECRLLRNLGADAEGMSTVPEVIVARHCGLRVFGFSLITNKVIMDYESQGKANHEEVLEAGKQAAQKLEQFVSLLMASIPVSGHTG

SEQ ID NO: 2 - protein, 277 aa, Artificial Sequence [sequence omitted]

SEQ ID NO: 3 - protein, 236 aa, Artificial Sequence
MTEFKQTPHINAKGEIAETVLLPGDPLRAKFIAERFLTDVVQFNSVRNMFGFTGTYNGKRISVMGTGMGMPSMGIYSYELIHVFGVKNLIRVGSCGALQDDLNLYDVILGMGASTNSNYVNQYHLPGTFAPLASYSLLEKAKKAADEKGVPVHVGNILSSDTFYNADEDAAGKWRDMGILGIEMEAAALYMNAAQAGVNALCILTVSDHIFKEEETTAEERETSFTNMMEIALELA

SEQ ID NO: 4 - protein, 292 aa, Artificial Sequence
MKKYFPSSELIINEDGSVFHLHVKPEWLADKVILVGDPGRVALVASHFENKECEVESREFKTVTGTYKGKRITVVSTGIGCDNIDIVVNELDALANIDFQTREEKEHLRSLELVRIGTCGGLQPNTPVGTFVCSEKSIGFDGLLNFYAGRNAVCDLPFERAFLNHMGWSGNMCAPAPYVIDANAELIDRIAQEDMVRGVTIAAGGFFGPQGRELRVPLADPKQNDKIEKFEYKGYKITNFEMESSALAGLSKLMGHKAMTVCMVIANRLIKEANTGYKNTIDTLIKTILDRI

SEQ ID NO: 5 - protein, 239 aa, Artificial Sequence
MATPHINAEMGDFADVVLMPGDPLRAKHIAETFLENVREVNNVRGMLGFTGTYKGRKISVMGHGMGIPSCSIYTKELITDFGVKKIIRVGSCGAVRMDVKLRDVVIGMGACTDSKVNRIRFKDHDFAAIADFDMVRNAVDAAKALGVDARVGNLFSADLFYSPDGEMFDVMEKYGVLGVEMEAAGIYGVAAEFGAKALTICTVSDHIRTHEQTTAAERQTTFNDMIKIALESVLLGDKE

SEQ ID NO: 6 - protein, 275 aa, Artificial Sequence
MQQDPVLNAVATILARKPGFAPRAAMILGSGLGVLADGLEEKVTIPYEELDGFPVSTVAGHSGELVLGKLHGVDVVCMKGRGHYYEHETMKVMTTPVRTFKRLGCELLLVTNAAGSLRPERIGVGSLVIFNDHINTMPGTPMTGANDEAYGPRFFSLANAYDKALRGEALALAEREGIAVNQGVFVSYSGPCFETAAEIRMMQIIGGDVVGMSVVPEVVSAAHCALPVLAICAITNMAEGLGDVQLSHEQTLKCAKLAETDFIRLINAFIKHHFQ

SEQ ID NO: 7 - protein, 305 aa, Artificial Sequence
MDIGELFGLAHVHEQRPLLHQLLPFGGGDFFHGGSIANPTEKKAGRAANRRKFGRNALRSPDTLRGMSIHLNAEKGQIAETVLLPGDPLRARHIAETFLENPVQHNTVRGMLGFTGTYKGERVSVQGTGMGIPSCMIYVNELIQDYGCKNLIRVGTAGSYQEGVHVRDLVLAQAACTDSNINRVRFGERTFAPIADFELLLRAYQIAQERGFSAHVGNIMSSDTFYNDNPTEFQRWAEFGVLAVEMEAAGLYTLAAKYGVRALTILTISDHLVTHEVTSAEERQLTFNGMIEVALDAALGLEKKA

SEQ ID NO: 8 - protein, 289 aa, Artificial Sequence
MENEFTYEDYQRTAEWLRSHTKHRPQVAVICGSGLGGLTAKLTQPQAFDYNEIPNFPQSTVQGHAGRLVFGFLNGRSCVMMQGRFHMYEGYSLSKVTFPVRVFHLLGVDTLVVTNAAGGLNPKFEVGDIMLIRDHINLPGFCGQNPLRGPNDERFGVRFPAMSDAYDRDMRQKAFNAWKQMGEQRELQEGTYIMSAGPTFETVAESCLLRMLGADAVGMSTVPEVIVARHCGLRVFGFSLITNKVVMDYNNLEKASHQEVLEAGKAAAQKLEQFVSILMESIPPRERAN

SEQ ID NO: 9 - protein, 421 aa, Artificial Sequence
MGFTTGREFHPALRMRAKYNAKYLGTKSEREKYFHLAYNKHTQFLRYQEQIMSKTKEKKVGVIFGKFYPVHTGHINMIYEAFSKVDELHVIVCSDTVRDLKLFYDSKMKRMPTVQDRLRWMQQIFKYQKNQIFIHHLVEDGIPSYPNGWQSWSEAVKTLFHEKHFEPSIVFSSEPQDKAPYEKYLGLEVSLVDPDRTFFNVSATKIRTTPFQYWKFIPKEARPFFAKTVAILGGESSGKSVLVNKLAAVFNTTSAWEYGREFVFEKLGGDEQAMQYSDYPQMALGHQRYIDYAVRHSHKIAFIDTDFITTQAFCIQYEGKAHPFLDSMIKEYPFDVTILLKNNTEWVDDGLRSLGSQKQRQQFQQLLKKLLDKYKVPYIEIESPSYLDRYNQVKAVIEKVLNEEEISELQNTTFPIKGTSQ

SEQ ID NO: 10 - protein, 410 aa, Artificial Sequence
MSSFDYLKTAIKQQGCTLQQVADASGMTKGYLSQLLNAKIKSPSAQKLEALHRFLGLEFPRRQKNIGVVFGKFYPLHTGHIYLIQRACSQVDELHIIMGYDDTRDRGLFEDSAMSQQPTVSDRLRWLLQTFKYQKNIRIHAFNEEGMEPYPHGWDVWSNGIKAFMAEKGIQPSWIYTSEEADAPQYLEHLGIETVLVDPERTFMNISGAQIRENPFRYWEYIPTEVKPFFVRTVAILGGESSGKSTLVNKLANIFNTTSAWEYGRDYVFSHLGGDEMALQYSDYDKIALGHAQYIDFAVKYANKVAFIDTDFVTTQAFCKKYEGREHPFVQALIDEYRFDLVILLENNTPWVADGLRSLGSSVDRKAFQNLLVEMLKENNIEFVHVKEADYDGRFLRCVELVKEMMGEQG

SEQ ID NO: 11 - protein, 200 aa, Artificial Sequence
MPEPGVGAHAGGLDADAALARFFVITGGPGSGKSTLIDALEARGYARSHEAGRGVIQDQVAIGGHALPWRDRAAFADMMLGWEMRSHHLARRARGPVFFDRGVPDVIGYLKLSALPVPAHLVAAAERFRYRRDVFIAPPWPEIYAQDAERRQDYAEAVRTYGAMVDTYAACGYRLIELPRASVDERCRFVLDVVEAAAAV

SEQ ID NO: 12 - protein, 240 aa, Artificial Sequence
MTSKKVILVALSGCSSSGKTTIAKLTASLFTKATLIHEDDFYKHDNEVPVDAKYNIQNWDSPEALDFKLFGKELDVIKQTGKIATKLIHNNNVDDPFTKFHIDRQVWDELKAKYDSINDDKYEVVIVDGFMIFNNTGISKKFDLKILVRAPYEVLKKRRASRKGYQTLDSFWVDPPYYFDEFVYESYRANHAQLFVNGDVEGLLDPRKSKNIKEFINDDDTPIAKPLSWVCQEILKLCKD

SEQ ID NO: 13 - protein, 241 aa, Artificial Sequence
MTSQLAGFKGTRGTLLVGIGGCSSSGKSTIAKLAVQVLEDAVLVHQDDFYRHDDEVPFDEEYQIGNWDVPEALDMAQFERELDHIRATGRPAAKLVHNGNIDDVGKFGISEEYLEELRRRYRGRISQPVVLVDGFMLYHDDKVAARFDCRLLVRAPYATMKARRASRGGYKTLDSFWQDPPFYFDKFVYKSYAATHARLFRNCDVEDRLVAPDVQEIYNGDEAQITCVLEQVLDAIAAAQC